European Patent Application EP 4 249 498 A1, published September 27, 2023. Title: Peptides and compositions for use in cosmetics and medicine. Applicant: Lipotrue S.L. The sequence listing filed with the application follows.

SEQUENCE LISTING (3 sequences)

SEQ ID NO: 1 - protein, 8 aa, Artificial Sequence
  Artificially synthesized sequence
  VARIANT 1: Xaa is a small amino acid
  VARIANT 2: Xaa is selected from polar uncharged or aromatic amino acids
  VARIANT 3: Xaa is absent or selected from aromatic amino acids
  VARIANT 4: Xaa is selected from negatively charged amino acids
  VARIANT 5: Xaa is selected from apolar amino acids
  VARIANT 6: Xaa is selected from Asn or Leu
  VARIANT 7: Xaa is selected from negatively charged amino acid
  VARIANT 8: Xaa is absent or selected from aromatic amino acids
XXXXXXXX

SEQ ID NO: 2 - protein, 7 aa, Artificial Sequence
  Artificially synthesized sequence
GYYELND

SEQ ID NO: 3 - protein, 7 aa, Artificial Sequence
  Artificially synthesized sequence
GNELLDY